European Patent Application EP 4 588 924 A1, published July 23, 2025. Title: MODIFIED OLIGONUCLEOTIDE PROBES FOR IN SITU HYBRIDIZATION. Applicant: Enzo Biochem, Inc. The sequence listing filed with the application follows.

SEQUENCE LISTING (68 sequences)

SEQ ID NO: 1 - DNA, 1181 bp, synthetic construct
  source 1..1181: mol_type = other DNA
ctacctgcgttcccgttccagcttccacttcagaatagccatatccactgtccgttagttccctggtttgaaacagccgtcgctttaccttttttggctgtcttgtaagtttaatggcgtccaatcgtggacttatttcactttccactgcctcggctatagtgtttataggactaacatatggactacctaaatactttcgttttaggtcctgcacagtcgcataatgggtgtccgcctcctgcctgttaaacaatgcctgtgcttccaaggaattgtgtgtaatattgctgtcatcaataaagtccaccatgtcatacccactgtcctccacctcctcatcctcatcgtctgatatttgtgtacctgttgggtgttgcactatagcttctaccataaaccatcctgtacacccagacccctcattttctgtacctgaatcgtccgccatcgttgttatgtcttcggtgcgcagatgggacacactatgtctagtgttcccaacagaagctgttgcacttctctgatgtctgtttctgtacactgcacaaccagtcgaacgttgctgtcacattcacagcaacaggtcactatttggaaatgttgttttaaaggttgtgaatcttgtccgtccacttcgtccacctcatcttctgagctgtctactaattgctcatagcaatgtaaccctacagggtctggaggttgcaggtctaatacaatatcctttagggtaacatgtcttccatgcatgttgtccagcagtgtaggcagcgacccttccacgtacaatttagctttataaaccgtgccttggttagtatatgttttaccttttctacttcacacagcggtttgtgacacaggtagcaccgaattagcacgtctaaaatgtcttgtttagtttcttcttcaacagttgttgcatatccagcataatcaaagtgtctatattggttgatttttccatgaaattctaggcagcacgcgcaggctgcatatggatagccgcctcgaaacaggacctttagctgtttatatgcatatgaataaatctctgcagtggtcagtgcattcttgcaaaacacacaattaatttgcaacgtatgcatagatagattaaacgtcttgcacaactggtctatggtcgttgcagacgtggaggcatttgcactttccat

SEQ ID NO: 2 - DNA, 1200 bp, synthetic construct
  source 1..1200: mol_type = other DNA
tttgaattcagtttccttcaagatcctcaagagagcttggttgggagcttctccactgggtgtaagaggctccacaagctccctctcctgcagcagcctccgcagcgtgcgcttccgaacgatgtggcgccttcgcatgaagaggccgatccccagggccaccaccagcagcaagaggagggcccccaccatcccagtggcgatggacgggatcttaggcccattcgttggacagccttcaagacctggcccagtgcatccgtaggtgcagtttggatggcacaggtggcacacatggccggcgtctgcgtacttccagaccagggtgttgttttctcccatgactcctgccgggcaggtcttgacgcagtgggggccgtcaatgtagtgggcacactggatacagttgtctggtccccgtcctgtgcaggtgatgttcatggcctgaggcaggcactctgggtggcactgtatgcactcagagttctccacaaactcccttggctcaccctccagaaggttgcacttgtccacgcattccctgcctcggctgacattccggcaagagacgcagtccctgggctccgggccccagcagccctcgggggagcacaaggcatggcagacctggcctgtggccttgcagctgttttcacctctgttgcttataattttggttttctgaccggaggtcccaaacagttttttccagtttattgtatttgcatagcacaaatttttgtttcctgaaattatcacatctccatcacttatctccttgagggagcgtaatcccaaggatgttatgttcaggctgacgactgcaagagaaaactgaccatgttgcttggtcctgccgcgtatgatttctaggttctcaaaggcatggaggtccgtcctgttttcaggccaagcctgaatcagcaaaaaccctgtgatttcctttacggttttcagaatatccagttcctgtggatccagaggaggagtatgtgtgaaggagtcacccctaaatgccaccggcaggatgtggagatcgccactgatggaggtgcagtttttgaagtgtttaatattcgtagcatttatggagagtgagtctttaaattcaccaatacctattccgttacacactttgcggcaaggcccttcgcacttcttacacttgcggacgccgtcttcctccatctcatagctgtc

SEQ ID NO: 3 - RNA, 30 nt, synthetic construct
  source 1..30: mol_type = other RNA
  misc_difference 1..30: note = 2-methoxy
agatcctcaagagagcttggttgggagctt

SEQ ID NO: 4 - RNA, 30 nt, synthetic construct
  source 1..30: mol_type = other RNA
  misc_difference 1..30: note = 2-methoxy
ctccactgggtgtaagaggctccacaagct

SEQ ID NO: 5 - RNA, 30 nt, synthetic construct
  source 1..30: mol_type = other RNA
  misc_difference 1..30: note = 2-methoxy
ttccgaacgatgtggcgccttcgcatgaag

SEQ ID NO: 6 - RNA, 30 nt, synthetic construct
  source 1..30: mol_type = other RNA
  misc_difference 1..30: note = 2-methoxy
cgatggacgggatcttaggcccattcgttg

SEQ ID NO: 7 - RNA, 30 nt, synthetic construct
  source 1..30: mol_type = other RNA
  misc_difference 1..30: note = 2-methoxy
ccagtgcatccgtaggtgcagtttggatgg

SEQ ID NO: 8 - RNA, 30 nt, synthetic construct
  source 1..30: mol_type = other RNA
  misc_difference 1..30: note = 2-methoxy
gtctgcgtacttccagaccagggtgttgtt

SEQ ID NO: 9 - RNA, 30 nt, synthetic construct
  source 1..30: mol_type = other RNA
  misc_difference 1..30: note = 2-methoxy
atacagttgtctggtccccgtcctgtgcag

SEQ ID NO: 10 - RNA, 30 nt, synthetic construct
  source 1..30: mol_type = other RNA
  misc_difference 1..30: note = 2-methoxy
gcactctgggtggcactgtatgcactcaga

SEQ ID NO: 11 - RNA, 30 nt, synthetic construct
  source 1..30: mol_type = other RNA
  misc_difference 1..30: note = 2-methoxy
ttggctcaccctccagaaggttgcacttgt

SEQ ID NO: 12 - RNA, 30 nt, synthetic construct
  source 1..30: mol_type = other RNA
  misc_difference 1..30: note = 2-methoxy
attttggttttctgaccggaggtcccaaac

SEQ ID NO: 13 - RNA, 30 nt, synthetic construct
  source 1..30: mol_type = other RNA
  misc_difference 1..30: note = 2-methoxy
ttatctccttgagggagcgtaatcccaagg

SEQ ID NO: 14 - RNA, 30 nt, synthetic construct
  source 1..30: mol_type = other RNA
  misc_difference 1..30: note = 2-methoxy
ggctgacgactgcaagagaaaactgaccat

SEQ ID NO: 15 - RNA, 30 nt, synthetic construct
  source 1..30: mol_type = other RNA
  misc_difference 1..30: note = 2-methoxy
gtcctgccgcgtatgatttctaggttctca

SEQ ID NO: 16 - RNA, 30 nt, synthetic construct
  source 1..30: mol_type = other RNA
  misc_difference 1..30: note = 2-methoxy
ggccaagcctgaatcagcaaaaaccctgtg

SEQ ID NO: 17 - RNA, 30 nt, synthetic construct
  source 1..30: mol_type = other RNA
  misc_difference 1..30: note = 2-methoxy
cagaatatccagttcctgtggatccagagg

SEQ ID NO: 18 - RNA, 30 nt, synthetic construct
  source 1..30: mol_type = other RNA
  misc_difference 1..30: note = 2-methoxy
ctaaatgccaccggcaggatgtggagatcg

SEQ ID NO: 19 - RNA, 30 nt, synthetic construct
  source 1..30: mol_type = other RNA
  misc_difference 1..30: note = 2-methoxy
ctattccgttacacactttgcggcaaggcc

SEQ ID NO: 20 - RNA, 30 nt, synthetic construct
  source 1..30: mol_type = other RNA
  misc_difference 1..30: note = 2-methoxy
tcgcacttcttacacttgcggacgccgtct

SEQ ID NO: 21 - RNA, 30 nt, synthetic construct
  source 1..30: mol_type = other RNA
  misc_difference 1..30: note = 2-methoxy
ggagggcttgcagagcatttatcagatggc

SEQ ID NO: 22 - RNA, 30 nt, synthetic construct
  source 1..30: mol_type = other RNA
  misc_difference 1..30: note = 2-methoxy
cacatttcctccaaaactctctgaggtggg

SEQ ID NO: 23 - RNA, 30 nt, synthetic construct
  source 1..30: mol_type = other RNA
  misc_difference 1..30: note = 2-methoxy
catgtgcttgtcaactgcggttgctccttc

SEQ ID NO: 24 - RNA, 30 nt, synthetic construct
  source 1..30: mol_type = other RNA
  misc_difference 1..30: note = 2-methoxy
agttgttgagcactctgtagggtcgagcag

SEQ ID NO: 25 - RNA, 30 nt, synthetic construct
  source 1..30: mol_type = other RNA
  misc_difference 1..30: note = 2-methoxy
attgactgtgaacttcgcccacaggcttct

SEQ ID NO: 26 - RNA, 30 nt, synthetic construct
  source 1..30: mol_type = other RNA
  misc_difference 1..30: note = 2-methoxy
ctctttgaaggcaggttgccactctttctc

SEQ ID NO: 27 - RNA, 30 nt, synthetic construct
  source 1..30: mol_type = other RNA
  misc_difference 1..30: note = 2-methoxy
ggcgttgatcactggcaactggagttttcc

SEQ ID NO: 28 - RNA, 30 nt, synthetic construct
  source 1..30: mol_type = other RNA
  misc_difference 1..30: note = 2-methoxy
caggtggagtgtgcattaccagagactttc

SEQ ID NO: 29 - RNA, 30 nt, synthetic construct
  source 1..30: mol_type = other RNA
  misc_difference 1..30: note = 2-methoxy
cccaccaaaggacacacgccttcttttcaa

SEQ ID NO: 30 - RNA, 30 nt, synthetic construct
  source 1..30: mol_type = other RNA
  misc_difference 1..30: note = 2-methoxy
agaagctagatcttgagacacgacgtgctg

SEQ ID NO: 31 - RNA, 30 nt, synthetic construct
  source 1..30: mol_type = other RNA
  misc_difference 1..30: note = 2-methoxy
caataccccttccaaacaagcaggtgctga

SEQ ID NO: 32 - RNA, 30 nt, synthetic construct
  source 1..30: mol_type = other RNA
  misc_difference 1..30: note = 2-methoxy
tcgaccccgctccttttgatagtaaccagg

SEQ ID NO: 33 - RNA, 30 nt, synthetic construct
  source 1..30: mol_type = other RNA
  misc_difference 1..30: note = 2-methoxy
cctcacagcggctcaactctcaaacttcca

SEQ ID NO: 34 - RNA, 30 nt, synthetic construct
  source 1..30: mol_type = other RNA
  misc_difference 1..30: note = 2-methoxy
cgatctctttgatgatggctgtcatgtctg

SEQ ID NO: 35 - RNA, 30 nt, synthetic construct
  source 1..30: mol_type = other RNA
  misc_difference 1..30: note = 2-methoxy
ctagctgtggtgggttatggtcttcaaaag

SEQ ID NO: 36 - RNA, 30 nt, synthetic construct
  source 1..30: mol_type = other RNA
  misc_difference 1..30: note = 2-methoxy
ccccatagaaatctagggcctcttgtgcct

SEQ ID NO: 37 - RNA, 30 nt, synthetic construct
  source 1..30: mol_type = other RNA
  misc_difference 1..30: note = 2-methoxy
acttgtcttcccgtcgtgtgggtcctgaat

SEQ ID NO: 38 - RNA, 30 nt, synthetic construct
  source 1..30: mol_type = other RNA
  misc_difference 1..30: note = 2-methoxy
tatcaccacacacaggtaacggctgaggga

SEQ ID NO: 39 - RNA, 30 nt, synthetic construct
  source 1..30: mol_type = other RNA
  misc_difference 1..30: note = 2-methoxy
tttctgaggtttcctctggtcctggtatga

SEQ ID NO: 40 - RNA, 30 nt, synthetic construct
  source 1..30: mol_type = other RNA
  misc_difference 1..30: note = 2-methoxy
cctctggatttgacggctcctctactgttt

SEQ ID NO: 41 - RNA, 30 nt, synthetic construct
  source 1..30: mol_type = other RNA
  misc_difference 1..30: note = 2-methoxy
cattctctggatcagagtcagtggtgtcag

SEQ ID NO: 42 - RNA, 30 nt, synthetic construct
  source 1..30: mol_type = other RNA
  misc_difference 1..30: note = 2-methoxy
gcattccctccattcccctaacccgaatac

SEQ ID NO: 43 - RNA, 30 nt, synthetic construct
  source 1..30: mol_type = other RNA
  misc_difference 1..30: note = 2-methoxy
acagcggccaattcctcgaatgtccagatt

SEQ ID NO: 44 - RNA, 30 nt, synthetic construct
  source 1..30: mol_type = other RNA
  misc_difference 1..30: note = 2-methoxy
gaagcttgcaggcagcacatgaagcatcca

SEQ ID NO: 45 - RNA, 30 nt, synthetic construct
  source 1..30: mol_type = other RNA
  misc_difference 1..30: note = 2-methoxy
tgaaattgaagccctagtcccaactcgggg

SEQ ID NO: 46 - RNA, 30 nt, synthetic construct
  source 1..30: mol_type = other RNA
  misc_difference 1..30: note = 2-methoxy
agaccacagctagtgaacaatttcagcacc

SEQ ID NO: 47 - RNA, 30 nt, synthetic construct
  source 1..30: mol_type = other RNA
  misc_difference 1..30: note = 2-methoxy
aaagcccccactttagtgcacagttccacc

SEQ ID NO: 48 - RNA, 30 nt, synthetic construct
  source 1..30: mol_type = other RNA
  misc_difference 1..30: note = 2-methoxy
cctcagtgcatagcatttacacacagagcc

SEQ ID NO: 49 - RNA, 30 nt, synthetic construct
  source 1..30: mol_type = other RNA
  misc_difference 1..30: note = 2-methoxy
gcttaacaaccagagtactaccaccaaagc

SEQ ID NO: 50 - RNA, 30 nt, synthetic construct
  source 1..30: mol_type = other RNA
  misc_difference 1..30: note = 2-methoxy
gacacacacacacacacttacaaactgcac

SEQ ID NO: 51 - RNA, 30 nt, synthetic construct
  source 1..30: mol_type = other RNA
  misc_difference 1..30: note = 2-methoxy
caggtaggtgagttccaggtttccctgcac

SEQ ID NO: 52 - RNA, 30 nt, synthetic construct
  source 1..30: mol_type = other RNA
  misc_difference 1..30: note = 2-methoxy
tgggacctgcctcacttggttgtgagcgat

SEQ ID NO: 53 - RNA, 30 nt, synthetic construct
  source 1..30: mol_type = other RNA
  misc_difference 1..30: note = 2-methoxy
cagtgtgagagccagctggttgttcttgtg

SEQ ID NO: 54 - RNA, 30 nt, synthetic construct
  source 1..30: mol_type = other RNA
  misc_difference 1..30: note = 2-methoxy
caggctctgacaatcctcagaactctctcc

SEQ ID NO: 55 - RNA, 30 nt, synthetic construct
  source 1..30: mol_type = other RNA
  misc_difference 1..30: note = 2-methoxy
aggcagtcacacagctggcgccgaatgtat

SEQ ID NO: 56 - RNA, 30 nt, synthetic construct
  source 1..30: mol_type = other RNA
  misc_difference 1..30: note = 2-methoxy
tggatattggcactggtaactgccctcacc

SEQ ID NO: 57 - RNA, 30 nt, synthetic construct
  source 1..30: mol_type = other RNA
  misc_difference 1..30: note = 2-methoxy
tccggccatgctgagatgtataggtaacct

SEQ ID NO: 58 - RNA, 30 nt, synthetic construct
  source 1..30: mol_type = other RNA
  misc_difference 1..30: note = 2-methoxy
gcagaattcgtccccggattacttgcaggt

SEQ ID NO: 59 - RNA, 30 nt, synthetic construct
  source 1..30: mol_type = other RNA
  misc_difference 1..30: note = 2-methoxy
acgaagcagaggtgggtgttatggtggatg

SEQ ID NO: 60 - RNA, 30 nt, synthetic construct
  source 1..30: mol_type = other RNA
  misc_difference 1..30: note = 2-methoxy
aaacagtgcctggcattcacatactccctg

SEQ ID NO: 61 - RNA, 30 nt, synthetic construct
  source 1..30: mol_type = other RNA
  misc_difference 1..30: note = 2-methoxy
gtccaaaacaggtcactgagccattctggg

SEQ ID NO: 62 - RNA, 30 nt, synthetic construct
  source 1..30: mol_type = other RNA
  misc_difference 1..30: note = 2-methoxy
catctggaaacttccagatgggcatgtagg

SEQ ID NO: 63 - RNA, 30 nt, synthetic construct
  source 1..30: mol_type = other RNA
  misc_difference 1..30: note = 2-methoxy
tgatgaggatcccaaagaccacccccaaga

SEQ ID NO: 64 - RNA, 30 nt, synthetic construct
  source 1..30: mol_type = other RNA
  misc_difference 1..30: note = 2-methoxy
tctctttcaggatccgcatctgcgcctggt

SEQ ID NO: 65 - RNA, 30 nt, synthetic construct
  source 1..30: mol_type = other RNA
  misc_difference 1..30: note = 2-methoxy
agctcatccccttggcaatctgcatacacc

SEQ ID NO: 66 - RNA, 30 nt, synthetic construct
  source 1..30: mol_type = other RNA
  misc_difference 1..30: note = 2-methoxy
tgtcatcgtcctccagcagtgagcggtaga

SEQ ID NO: 67 - RNA, 30 nt, synthetic construct
  source 1..30: mol_type = other RNA
  misc_difference 1..30: note = 2-methoxy
gtactgtggggtcctcactgtaccgctgta

SEQ ID NO: 68 - RNA, 30 nt, synthetic construct
  source 1..30: mol_type = other RNA
  misc_difference 1..30: note = 2-methoxy
gttcttagacactcccttagggccgcttcc